European Patent Application EP 4 335 860 A1, published March 13, 2024. Title: Peptides having blood coagulation activity and use thereof. Applicant: CAREGEN CO., LTD. The sequence listing filed with the application follows.

SEQUENCE LISTING (1 sequence)

SEQ ID NO: 1 - protein, 12 aa, Artificial Sequence
  peptide having blood coagulation activity
SASQAYLAGNIT